European Patent Application EP 4 667 574 A1, published December 24, 2025. Title: CONSTRUCTION OF PLASMID EXPRESSION VECTOR BASED ON TAC PROMOTER AND USES THEREOF. Applicant: BEIJING HEALTH GUARD BIOTECHNOLOGY, INC. The sequence listing filed with the application follows.

SEQUENCE LISTING (16 sequences)

SEQ ID NO: 1 - protein, 469 aa, synthetic construct
MPSDSTVYVPPPNPVSKVVATDAYVTRTNIFYHASSSRLLAVGHPYFSIKRANKTVVPKVSGYQYRVFKVVLPDPNKFALPDSSLFDPTTQRLVWACTGLEVGRGQPLGVGVSGHPFLNKYDDVENSGSGGNPGQDNRVNVGMDYKQTQLCMVGCAPPLGEHWGKGKQCTNTPVQAGDCPPLELITSVIQDGDMVDTGFGAMNFADLQTNKSDVPIDICGTTCKYPDYLQMAADPYGDRLFFFLRKEQMFARHFFNRAGEVGEPVPDTLIIKGSGNRTSVGSSIYVNTPSGSLVSSEAQLFNKPYWLQKAQGHNNGICWGNQLFVTVVDTTRSTNMTLCASVTTSSTYTNSDYKEYMRHVEEYDLQFIFQLCSITLSAEVMAYIHTMNPSVLEDWNFGLSPPPNGTLEDTYRYVQSQAITCQKPTPEKEKPDPYKNLSFWEVNLKEKFSSELDQYPLGRKFLLQSGYRG

SEQ ID NO: 2 - protein, 470 aa, synthetic construct
MPSDSTVYVPPPNPVSKVVATDAYVKRTNIFYHASSSRLLAVGHPYYSIKKVNKTVVPKVSGYQYRVFKVVLPDPNKFALPDSSLFDPTTQRLVWACTGLEVGRGQPLGVGVSGHPLLNKYDDVENSGGYGGNPGQDNRVNVGMDYKQTQLCMVGCAPPLGEHWGKGTQCSNTSVQNGDCPPLELITSVIQDGDMVDTGFGAMNFADLQTNKSDVPLDICGTVCKYPDYLQMAADPYGDRLFFYLRKEQMFARHFFNRAGTVGEPVPDDLLVKGGNNRSSVASSIYVHTPSGSLVSSEAQLFNKPYWLQKAQGHNNGICWGNHLFVTVVDTTRSTNMTLCASVSKSATYTNSDYKEYMRHVEEFDLQFIFQLCSITLSAEVMAYIHTMNPSVLEDWNFGLSPPPNGTLEDTYRYVQSQAITCQKPTPEKEKQDPYKDMSFWEVNLKEKFSSELDQFPLGRKFLLQSGYRG

SEQ ID NO: 3 - protein, 472 aa, synthetic construct
MPSEATVYLPPVPVSKVVSTDEYVARTNIYYHAGTSRLLAVGHPYFPIKKPNNNKILVPKVSGLQYRVFRIHLPDPNKFGFPDTSFYNPDTQRLVWACVGVEVGRGQPLGVGISGHPLLNKLDDTENASAYAANAGVDNRECISMDYKQTQLCLIGCKPPIGEHWGKGSPCTNVAVNPGDCPPLELINTVIQDGDMVDTGFGAMDFTTLQANKSEVPLDICTSICKYPDYIKMVSEPYGDSLFFYLRREQMFVRHLFNRAGAVGENVPDDLYIKGSGSTANLASSNYFPTPSGSMVTSDAQIFNKPYWLQRAQGHNNGICWGNQLFVTVVDTTRSTNMSLCAAISTSETTYKNTNFKEYLRHGEEYDLQFIFQLCKITLTADVMTYIHSMNSTILEDWNFGLQPPPGGTLEDTYRFVTSQAIACQKHTPPAPKEDPLKKYTFWEVNLKEKFSADLDQFPLGRKFLLQAGLKA

SEQ ID NO: 4 - protein, 473 aa, synthetic construct
MPSDNTVYLPPPSVARVVNTDDYVTRTSIFYHAGSSRLLTVGNPYFRVPAGGGNKQDIPKVSAYQYRVFRVQLPDPNKFGLPDNSIYNPETQRLVWACAGVEIGRGQPLGVGLSGHPFYNKLDDTESSHAATSNVSEDVRDNVSVDYKQTQLCILGCAPAIGEHWAKGTACKSRPLSQGDCPPLELKNTVLEDGDMVDTGYGAMDFSTLQDTKCEVPLDICQSICKYPDYLQMSADPYGDSMFFCLRREQLFARHFWNRAGTMGDTVPQSLYIKGTGMRASPGSCVYSPSPSGSIVTSDSQLFNKPYWLHKAQGHNNGVCWHNQLFVTVVDTTRSTNLTICASTQSPVPGQYDATKFKQYSRHVEEYDLQFIFQLCTITLTADVMSYIHSMNSSILEDWNFGVPPPPTTSLVDTYRFVQSVAITCQKDAAPAENKDPYDKLKFWNVDLKEKFSLDLDQYPLGRKFLVQAGLRR

SEQ ID NO: 5 - protein, 473 aa, synthetic construct
MPSEATVYLPPVPVSKVVSTDEYVTRTNIYYHAGSARLLTVGHPYYSIPKSDNPKKIVVPKVSGLQYRVFRVRLPDPNKFGFPDTSFYNPETQRLVWACVGLEVGRGQPLGVGISGHPLLNKFDDTENSNRYAGGPGTDNRECISMDYKQTQLCLLGCKPPIGEHWGKGSPCSNNAITPGDCPPLELKNSVIQDGDMVDTGFGAMDFTALQDTKSNVPLDICNSICKYPDYLKMVAEPYGDTLFFYLRREQMFVRHFFNRSGTVGESVPTDLYIKGSGSTATLANSTYFPTPSGSMVTSDAQIFNKPYWMQRAQGHNNGICWGNQLFVTVVDTTRSTNMSVCAAIANSDTTFKSSNFKEYLRHGEEFDLQFIFQLCKITLSADIMTYIHSMNPAILEDWNFGLTTPPSGSLEDTYRFVTSQAITCQKTAPQKPKEDPFKDYVFWEVNLKEKFSADLDQFPLGRKFLLQAGYRA

SEQ ID NO: 6 - protein, 471 aa, synthetic construct
MPSEATVYLPPVPVSKVVSTDEYVSRTSIYYYAGSSRLLAVGHPYFSIKNPNNAKKLLVPKVSGLQYRVFRVRLPDPNKFGFPDTSFYNPDTQRLVWACVGLEIGRGQPLGVGISGHPLLNKFDDTETSNKYPGQPGADNRECLSMDYKQTQLCLLGCKPPTGEHWGKGVACTNAAPANDCPPLELINTIIEDGDMVDTGFGCMDFKTLQANKSDVPIDICGSTCKYPDYLKMTSEPYGDSLFFFLRREQMFVRHFFNRAGKLGEAVPDDLYIKGSGTTASIQSSAFFPTPSGSMVTSESQLFNKPYWLQRAQGHNNGICWGNQVFVTVVDTTRSTNMTLCTQVTSDSTYKNENFKEYIRHVEEYDLQFVFQLCKVTLTAEVMTYIHAMNPDILEDWQFGLTPPPSASLQDTYRFVTSQAITCQKTVPPKEKEDPLGKYTFWEVDLKEKFSADLDQFPLGRKFLLQAGLKA

SEQ ID NO: 7 - protein, 470 aa, synthetic construct
MSNEATVYLPPVSVSKVVSTDEYVTRTNIYYHAGSSRLLAVGHPYYAIKKQDSNKIAVPKVSGLQYRVFRVKLPDPNKFGFPDTSFYDPASQRLVWACTGVEVGRGQPLGVGISGHPLLNKLDDTENSNKYVGNSGTDNRECISMDYKQTQLCLIGCRPPIGEHWGKGTPCNANQVKAGECPPLELLNTVLQDGDMVDTGFGAMDFTTLQANKSDVPLDICSSICKYPDYLKMVSEPYGDMLFFYLRREQMFVRHLFNRAGTVGETVPADLYIKGTTGTLPSTSYFPTPSGSMVTSDAQIFNKPYWLQRAQGHNNGICWSNQLFVTVVDTTRSTNMSVCSAVSTSDSTYKNDNFKEYLRHGEEYDLQFIFQLCKITLTADVMTYIHSMNPSILEDWNFGLTPPPSGTLEDTYRYVTSQAVTCQKPSAPKPKDDPLKNYTFWEVDLKEKFSADLDQFPLGRKFLLQAGLKA

SEQ ID NO: 8 - protein, 467 aa, synthetic construct
MVYLPPPSVAKVVNTDDYVTRTGIYYYAGSSRLLTVGHPYFKVGMNGGRKQDIPKVSAYQYRVFRVTLPDPNKFSIPDASLYNPETQRLVWACVGVEVGRGQPLGVGISGHPLYNRQDDTENSPFSSTTNKDSRDNVSVDYKQTQLCIIGCVPAIGEHWGKGKACKPNNVSTGDCPPLELVNTPIEDGDMIDTGYGAMDFGALQETKSEVPLDICQSICKYPDYLQMSADVYGDSMFFCLRREQLFARHFWNRGGMVGDAIPAQLYIKGTDIRANPGSSVYCPSPSGSMVTSDSQLFNKPYWLHKAQGHNNGICWHNQLFLTVVDTTRSTNFTLSTSIESSIPSTYDPSKFKEYTRHVEEYDLQFIFQLCTVTLTTDVMSYIHTMNSSILDNWNFAVAPPPSASLVDTYRYLQSAAITCQKDAPAPEKKDPYDGLKFWNVDLREKFSLELDQFPLGRKFLLQARVRR

SEQ ID NO: 9 - protein, 476 aa, synthetic construct
MPSDSTVYLPPPSVARVVNTDDYVSRTSIFYHAGSSRLLTVGNPYFRVVPNGAGNKQAVPKVSAYQYRVFRVALPDPNKFGLPDSTIYNPETQRLVWACVGMEIGRGQPLGIGLSGHPFYNKLDDTESAHAATAVITQDVRDNVSVDYKQTQLCILGCVPAIGEHWAKGTLCKPAQLQPGDCPPLELKNTIIEDGDMVDTGYGAMDFSTLQDTKCEVPLDICQSICKYPDYLQMSADPYGDSMFFCLRREQLFARHFWNRAGVMGDTVPTDLYIKGTSANMRETPGSCVYSPSPSGSIITSDSQLFNKPYWLHKAQGHNNGICWHNQLFVTVVDTTRSTNLTLCASTQNPVPSTYDPTKFKQYSRHVEEYDLQFIFQLCTITLTAEVMSYIHSMNSSILENWNFGVPPPPTTSLVDTYRFVQSVAVTCQKDTTPPEKQDPYDKLKFWTVDLKEKFSSDLDQYPLGRKFLVQAGLRR

SEQ ID NO: 10 - protein, 472 aa, synthetic construct
MTNDSKVYLPPAPVSRIVNTEEYITRTGIYYYAGSSRLITLGHPYFPIPKTSTRAAIPKVSAFQYRVFRVQLPDPNKFGLPDPNLYNPDTDRLVWGCVGVEVGRGQPLGVGLSGHPLFNKYDDTENSRIANGNAQQDVRDNTSVDNKQTQLCIIGCAPPIGEHWGIGTTCKNTPVPPGDCPPLELVSSVIQDGDMIDTGFGAMDFAALQATKSDVPLDISQSVCKYPDYLKMSADTYGNSMFFHLRREQIFARHYYNKLGSVGEDIPNDYYIKGSGNGRDPIESYIYSATPSGSMITSDSQIFNKPYWLHRAQGHNNGICWNNQLFITCVDTTRSTNLTISTATAAVSPTFTPSNFKQYIRHGEEYELQFIFQLCKITLTTEVMAYLHTMDPTILEQWNFGLTLPPSASLEDAYRFVTNAATSCQKDTPPQAKPDPLAKYKFWDVDLKERFSLDLDQFALGRKFLLQVGVQR

SEQ ID NO: 11 - protein, 476 aa, synthetic construct
MPSEATVYLPPVPVSKVVSTDEYVSRTSIYYYAGSSRLLTVGHPYFSIKNTSSGNGKKVLVPKVSGLQYRVFRIKLPDPNKFGFPDTSFYNPETQRLVWACTGLEIGRGQPLGVGISGHPLLNKFDDTETSNKYAGKPGIDNRECLSMDYKQTQLCILGCKPPIGEHWGKGTPCNNNSGNPGDCPPLQLINSVIQDGDMVDTGFGCMDFNTLQASKSDVPIDICSSVCKYPDYLQMASEPYGDSLFFFLRREQMFVRHFFNRAGTLGDPVPGDLYIQGSNSGNTATVQSSAFFPTPSGSMVTSESQLFNKPYWLQRAQGHNNGICWGNQLFVTVVDTTRSTNMTLCAEVKKESTYKNENFKEYLRHGEEFDLQFIFQLCKITLTADVMTYIHKMDATILEDWQFGLTPPPSASLEDTYRFVTSTAITCQKNTPPKGKEDPLKDYMFWEVDLKEKFSADLDQFPLGRKFLLQAGLQA

SEQ ID NO: 12 - protein, 470 aa, synthetic construct
MPSENKVYLPPTPVSKVVATDSYVKRTSIFYHAGSSRLLAVGHPYYSVTKDNTKTNIPKVSAYQYRVFRVRLPDPNKFGLPDTNIYNPDQERLVWACVGLEVGRGQPLGAGLSGHPLFNRLDDTESSNLANNNVIEDSRDNISVDGKQTQLCIVGCTPAMGEHWTKGAVCKSTQVTTGDCPPLALINTPIEDGDMIDTGFGAMDFKVLQESKAEVPLDIVQSTCKYPDYLKMSADAYGDSMWFYLRREQLFARHYFNRAGKVGETIPAELYLKGSNGREPPPSSVYVATPSGSMITSEAQLFNKPYWLQRAQGHNNGICWGNQLFVTVVDTTRSTNMTISTATEQLSKYDARKINQYLRHVEEYELQFVFQLCKITLSAEVMAYLHNMNANLLEDWNIGLSPPVATSLEDKYRYVTSTAITCQREQPPTEKQDPLAKYKFWDVNLQDSFSTDLDQFPLGRKFLMQLGTRS

SEQ ID NO: 13 - protein, 471 aa, synthetic construct
MPSEATVYLPPVPVSKVVSTDEYVSRTSIYYYAGSSRLLAVGNPYFSIKSPNNNKKVLVPKVSGLQYRVFRVRLPDPNKFGFPDTSFYNPDTQRLVWACVGLEIGRGQPLGVGVSGHPYFNKFDDTETSNRYPAQPGSDNRECLSMDYKQTQLCLIGCKPPTGEHWGKGVACNNNAAATDCPPLELFNSIIEDGDMVDTGFGCMDFGTLQANKSDVPIDICNSTCKYPDYLKMASEPYGDSLFFFLRREQMFVRHFFNRAGKLGEAVPDDLYIKGSGNTAVIQSSAFFPTPSGSMVTSESQLFNKPYWLQRAQGHNNGICWGNQLFVTVVDTTRSTNMTLCTEVTKEGTYKNDNFKEYVRHVEEYDLQFVFQLCKITLTAEIMTYIHTMDSNILEDWQFGLTPPPSASLQDTYRFVTSQAITCQKTAPPKEKEDPLNKYTFWEVNLKEKFSADLDQFPLGRKFLLQSGLKA

SEQ ID NO: 14 - protein, 473 aa, synthetic construct
MSSDNKVYLPPPSVAKVVSTDEYVTRTSIFYHAGSSRLLTVGHPYFKVPKGGNGRQDVPKVSAYQYRVFRVKLPDPNKFGLPDNTVYDPNSQRLVWACVGVEIGRGQPLGVGLSGHPLYNKLDDTENSHVASAVDTKDTRDNVSVDYKQTQLCIIGCVPAIGEHWTKGTACKPTTVVQGDCPPLELINTPIEDGDMVDTGYGAMDFKLLQDNKSEVPLDICQSICKYPDYLQMSADAYGDSMFFCLRREQVFARHFWNRSGTMGDQLPESLYIKGTDIRANPGSYLYSPSPSGSVVTSDSQLFNKPYWLHKAQGLNNGICWHNQLFLTVVDTTRSTNLSVCASTTSSIPNVYTPTSFKEYARHVEEFDLQFIFQLCKITLTTEVMSYIHNMNTTILEDWNFGVTPPPTASLVDTYRFVQSAAVTCQKDTAPPVKQDPYDKLKFWPVDLKERFSADLDQFPLGRKFLLQLGARP

SEQ ID NO: 15 - protein, 473 aa, synthetic construct
MASDNMVYLPPPSVAKVVNTDDYVTRTGMYYYAGTSRLLTVGHPYFKVPMSGGRKQGIPKVSAYQYRVFRVTLPDPNKFSVPESTLYNPDTQRMVWACVGVEIGRGQPLGVGLSGHPLYNRLDDTENSPFSSNKNPKDSRDNVAVDCKQTQLCIIGCVPAIGEHWAKGKSCKPTNVQQGDCPPLELVNTPIEDGDMIDTGYGAMDFGTLQETKSEVPLDICQSVCKYPDYLQMSADVYGDSMFFCLRREQLFARHFWNRGGMVGDTIPTDMYIKGTDIRETPSSYVYAPSPSGSMVSSDSQLFNKPYWLHKAQGHNNGICWHNQLFLTVVDTTRSTNFTLSTTTDSTVPAVYDSNKFKEYVRHVEEYDLQFIFQLCTITLSTDVMSYIHTMNPAILDDWNFGVAPPPSASLVDTYRYLQSAAITCQKDAPAPVKKDPYDGLNFWNVDLKEKFSSELDQFPLGRKFLLQAGVRR

SEQ ID NO: 16 - DNA, 552 bp, Human rhinovirus
  source 1..552: mol_type = other DNA
atgggaccaaacacagaatttgcactatccctgttaaggaaaaacataatgactataacaacctcaaagggagagttcacagggttaggcatacatgatcgtgtctgtgtgatacccacacacgcacagcctggtgatgatgtactagtgaatggtcagaaaattagagttaaggataagtacaaattagtagatccagagaacattaatctagagcttacagtgttgactttagatagaaatgaaaaattcagagatatcaggggatttatatcagaagatctagaaggtgtggatgccactttggtagtacattcaaataactttaccaacactatcttagaagttggccctgtaacaatggcaggacttattaatttgagtagcacccccactaacagaatgattcgttatgattatgcaacaaaaactgggcagtgtggaggtgtgctgtgtgctactggtaagatctttggtattcatgttggcggtaatggaagacaaggattttcagctcaacttaaaaaacaatattttgtagagaaacaataa